European Patent Specification EP 3 880 847 B1, published September 3, 2025. Title: METHODS AND COMPOSITIONS FOR CHARACTERIZING BLADDER CANCER. Applicant: OSLO UNIVERSITETSSYKEHUS HF. The sequence listing filed with the application follows.

SEQUENCE LISTING (28 sequences)

SEQ ID NO: 1 - DNA, 200 bp, Homo sapiens
ggcgcgggcactggatgctagccgttttgctccaggagatataagaagcccaggttttcccccttcctgggagcgctgcggatcattcgcaggcggcccggcaccctcgcataggtgggccggcccctggggctccagccgtgcgaccccggaaccacacgtgtggcgaggaacgggtcccggggcggagtaggcagagt

SEQ ID NO: 2 - DNA, 400 bp, Homo sapiens
agtgggtgaactgctcccgctccgcctcgctcagcagcgcggtcagcgcttggtgcagctggcgcacgttggcagacagtaaccgcagccccgcgcccccgccgccgcccgccccggccgccgagcccagcgagccggtggaggacgagctcaccgacaggccgtccagcggcgcgttcatctccacgccgaggcccggccgggctctgagcgcgcggggtgtgggcggtgccgctgtcctcgcgggtactggcgcgacagctggatccccgggagcgcggagacgacggctggagcctgggtttggggagcacgggtacagtggctggatcctagggggtcgcggagaccgctgctagagtcccggaggcgcgaagacggcgggggtcgcgaacctgga

SEQ ID NO: 3 - DNA, 1000 bp, Homo sapiens
ccctagcgcccgggctccacgggccgcgcccccacgcggcgcctcccagagaccctcctccctccgggtgggcggcgcagcggggcctcggcgccgcgaggaccccccgcgccagaacaaaggaatgtggggagggggcagggaggagctcaggccactgagcagccccagtataactgccgttcggaggcgcttctcggtcccgacccgaggtccccgcccgccactaccagacccgcccccagccccggattctcgcagaccccaccggcccgcaggagggagcggcgcactgggggccgcacggactcgccattggagatcgcgatcggaaggtggcgccacgcggcccctacaggcctgggactcccacccgagctcgcaaagtaggtcggggtctgaagctgggggcctagagcaactagcttcttggaaagcgactgcaattatttggggtaatatactctgttccagagacgtccaccccccacctcccacaaaaaaaaaccctgcacttaatttaaatgttacgttatatatacatcccatcatatacatatattcacacataatcactatgtaacagtccaggaagaaatttaatatttgggtaaattacatattcacacatcttcacataagtaaaaccagggtatccagacaaaaaaacaatctactaacctatatctgtttcccataggtcatatctggtctgggggtaaataaatacttctgacctcacttactgttgttatttacaaaagccaagaacagaagatgacacttggccattccctgctgttctcagagaacagcagtttcctaaagtgtcctttaaaaacataaatgggagccagcatccagcaaatcaccgggcgctgcgaaatgccttcctaaaaatacaatcttatcaaaggtctccgaaggcgtggagttaaaactacagcaaatggccttgaacttgtatttgcacacagccctggagaaaacaccagaaata

SEQ ID NO: 4 - DNA, 200 bp, Homo sapiens
gcaacagcgtggggtccggtcggcagtggggcgcgggctgcgcggtaagcagctcctcggagctcagcaccagccccagcactatgcagggtacccacgaggcggaggccagcaggcgccgggcccggccaaagccgcccgcagctctcagcacccgcgcctcctgctccatcggtcgcaggctgcgctcgggacggggc

SEQ ID NO: 5 - DNA, 200 bp, Homo sapiens
gtccgcgcgggcggggcgaggtcggggagggcagctgcccgccctcctcggcactgggagctttcggctggtactgcgggaggagctcccgggtgacccgcgggttctgaaaccgccgctcgggagctcggggcctgcgcggcgtctacggggcgagcgagggagaactgacgcctttcgctcggatccttctccccttc

SEQ ID NO: 6 - DNA, 300 bp, Homo sapiens
cgggtgccgcggcgggcgcctcgcagcgcggcccggtccagccctgcgcgcaagcgcagcggaagaagggcgcgagcggcgcggggcggcaggagcccccgtggagacagggggcggccgcgcagctggcgttgctggcccccggcggcgaccccgggaagctgcggcaggagggtcccgacaaccctggggggcaggcgcagcgcggcccgcggggcgtctgctggcatgggacgcccaccgggcactgcagctcccggcaggagcgcgccacccgctcgcaacgcggaccccagaacg

SEQ ID NO: 7 - DNA, 300 bp, Homo sapiens
gcgagggaagggggcagccggcggtgagcaggggcgtttgttattttgctccacgcctgggcagagccacgccccttgtcgcgctattggtggagtcccttcccggggcggggaagagacggtgaccccacccccccccgccctgccgtataaaagcggcgccgacgcacggcgcggggattttctgctccggttggtgagcgcgcctgcgcgttgacggcgattttgcgttctgaggctgcagcgtcggcatcttgagctgccggttcgcgagttcgaggccaggttccgcctgtcgtg

SEQ ID NO: 8 - DNA, 200 bp, Artificial sequence
  Synthetic
ggcgcgggtattggatgttagtcgttttgttttaggagatataagaagtttaggttttttttttttttgggagcgttgcggattattcgtaggcggttcggtattttcgtataggtgggtcggtttttggggttttagtcgtgcgatttcggaattatacgtgtggcgaggaacgggtttcggggcggagtaggtagagt

SEQ ID NO: 9 - DNA, 400 bp, Artificial sequence
  Synthetic
agtgggtgaattgttttcgtttcgtttcgtttagtagcgcggttagcgtttggtgtagttggcgtacgttggtagatagtaatcgtagtttcgcgttttcgtcgtcgttcgtttcggtcgtcgagtttagcgagtcggtggaggacgagtttatcgataggtcgtttagcggcgcgtttatttttacgtcgaggttcggtcgggttttgagcgcgcggggtgtgggcggtgtcgttgttttcgcgggtattggcgcgatagttggattttcgggagcgcggagacgacggttggagtttgggtttggggagtacgggtatagtggttggattttagggggtcgcggagatcgttgttagagtttcggaggcgcgaagacggcgggggtcgcgaatttgga

SEQ ID NO: 10 - DNA, 1000 bp, Artificial sequence
  Synthetic
ttttagcgttcgggttttacgggtcgcgtttttacgcggcgttttttagagattttttttttttcgggtgggcggcgtagcggggtttcggcgtcgcgaggatttttcgcgttagaataaaggaatgtggggagggggtagggaggagtttaggttattgagtagttttagtataattgtcgttcggaggcgtttttcggtttcgattcgaggttttcgttcgttattattagattcgtttttagtttcggattttcgtagattttatcggttcgtaggagggagcggcgtattgggggtcgtacggattcgttattggagatcgcgatcggaaggtggcgttacgcggtttttataggtttgggatttttattcgagttcgtaaagtaggtcggggtttgaagttgggggtttagagtaattagttttttggaaagcgattgtaattatttggggtaatatattttgttttagagacgtttattttttattttttataaaaaaaaattttgtatttaatttaaatgttacgttatatatatattttattatatatatatatttatatataattattatgtaatagtttaggaagaaatttaatatttgggtaaattatatatttatatatttttatataagtaaaattagggtatttagataaaaaaataatttattaatttatatttgttttttataggttatatttggtttgggggtaaataaatatttttgattttatttattgttgttatttataaaagttaagaatagaagatgatatttggttattttttgttgtttttagagaatagtagttttttaaagtgttttttaaaaatataaatgggagttagtatttagtaaattatcgggcgttgcgaaatgtttttttaaaaatataattttattaaaggttttcgaaggcgtggagttaaaattatagtaaatggttttgaatttgtatttgtatatagttttggagaaaatattagaaata

SEQ ID NO: 11 - DNA, 200 bp, Artificial sequence
  Synthetic
gtaatagcgtggggttcggtcggtagtggggcgcgggttgcgcggtaagtagtttttcggagtttagtattagttttagtattatgtagggtatttacgaggcggaggttagtaggcgtcgggttcggttaaagtcgttcgtagtttttagtattcgcgttttttgttttatcggtcgtaggttgcgttcgggacggggc

SEQ ID NO: 12 - DNA, 200 bp, Artificial sequence
  Synthetic
gttcgcgcgggcggggcgaggtcggggagggtagttgttcgtttttttcggtattgggagttttcggttggtattgcgggaggagttttcgggtgattcgcgggttttgaaatcgtcgttcgggagttcggggtttgcgcggcgtttacggggcgagcgagggagaattgacgtttttcgttcggatttttttttttttt

SEQ ID NO: 13 - DNA, 300 bp, Artificial sequence
  Synthetic
cgggtgtcgcggcgggcgtttcgtagcgcggttcggtttagttttgcgcgtaagcgtagcggaagaagggcgcgagcggcgcggggcggtaggagttttcgtggagatagggggcggtcgcgtagttggcgttgttggttttcggcggcgatttcgggaagttgcggtaggagggtttcgataattttggggggtaggcgtagcgcggttcgcggggcgtttgttggtatgggacgtttatcgggtattgtagttttcggtaggagcgcgttattcgttcgtaacgcggattttagaacg

SEQ ID NO: 14 - DNA, 300 bp, Artificial sequence
  Synthetic
gcgagggaagggggtagtcggcggtgagtaggggcgtttgttattttgttttacgtttgggtagagttacgttttttgtcgcgttattggtggagttttttttcggggcggggaagagacggtgattttattttttttcgttttgtcgtataaaagcggcgtcgacgtacggcgcggggattttttgtttcggttggtgagcgcgtttgcgcgttgacggcgattttgcgttttgaggttgtagcgtcggtattttgagttgtcggttcgcgagttcgaggttaggtttcgtttgtcgtg

SEQ ID NO: 15 - DNA, 89 bp, Artificial sequence
  Synthetic
cccccttcctgggagcgctgcggatcattcgcaggcggcccggcaccctcgcataggtgggccggcccctggggctccagccgtgcgac

SEQ ID NO: 16 - DNA, 111 bp, Artificial sequence
  Synthetic
ggaggacgagctcaccgacaggccgtccagcggcgcgttcatctccacgccgaggcccggccgggctctgagcgcgcggggtgtgggcggtgccgctgtcctcgcgggtac

SEQ ID NO: 17 - DNA, 91 bp, Artificial sequence
  Synthetic
cgcgcccccacgcggcgcctcccagagaccctcctccctccgggtgggcggcgcagcggggcctcggcgccgcgaggaccccccgcgccag

SEQ ID NO: 18 - DNA, 95 bp, Artificial sequence
  Synthetic
cagtggggcgcgggctgcgcggtaagcagctcctcggagctcagcaccagccccagcactatgcagggtacccacgaggcggaggccagcaggcg

SEQ ID NO: 19 - DNA, 107 bp, Artificial sequence
  Synthetic
ggagggcagctgcccgccctcctcggcactgggagctttcggctggtactgcgggaggagctcccgggtgacccgcgggttctgaaaccgccgctcgggagctcggg

SEQ ID NO: 20 - DNA, 110 bp, Artificial sequence
  Synthetic
gcggccgcgcagctggcgttgctggcccccggcggcgaccccgggaagctgcggcaggagggtcccgacaaccctggggggcaggcgcagcgcggcccgcggggcgtctg

SEQ ID NO: 21 - DNA, 132 bp, Artificial sequence
  Synthetic
caggggcgtttgttattttgctccacgcctgggcagagccacgccccttgtcgcgctattggtggagtcccttcccggggcggggaagagacggtgaccccacccccccccgccctgccgtataaaagcggc

SEQ ID NO: 22 - DNA, 88 bp, Artificial sequence
  Synthetic
ttttttttttgggagcgttgcggattattcgtaggcggttcggtattttcgtataggtgggtcggtttttggggttttagtcgtgcga

SEQ ID NO: 23 - DNA, 111 bp, Artificial sequence
  Synthetic
ggaggacgagtttatcgataggtcgtttagcggcgcgtttatttttacgtcgaggttcggtcgggttttgagcgcgcggggtgtgggcggtgtcgttgttttcgcgggtat

SEQ ID NO: 24 - DNA, 91 bp, Artificial sequence
  Synthetic
cgcgtttttacgcggcgttttttagagattttttttttttcgggtgggcggcgtagcggggtttcggcgtcgcgaggatttttcgcgttag

SEQ ID NO: 25 - DNA, 95 bp, Artificial sequence
  Synthetic
tagtggggcgcgggttgcgcggtaagtagtttttcggagtttagtattagttttagtattatgtagggtatttacgaggcggaggttagtaggcg

SEQ ID NO: 26 - DNA, 107 bp, Artificial sequence
  Synthetic
ggagggtagttgttcgtttttttcggtattgggagttttcggttggtattgcgggaggagttttcgggtgattcgcgggttttgaaatcgtcgttcgggagttcggg

SEQ ID NO: 27 - DNA, 110 bp, Artificial sequence
  Synthetic
gcggtcgcgtagttggcgttgttggttttcggcggcgatttcgggaagttgcggtaggagggtttcgataattttggggggtaggcgtagcgcggttcgcggggcgtttg

SEQ ID NO: 28 - DNA, 132 bp, Artificial sequence
  Synthetic
taggggcgtttgttattttgttttacgtttgggtagagttacgttttttgtcgcgttattggtggagttttttttcggggcggggaagagacggtgattttattttttttcgttttgtcgtataaaagcggc